European Patent Specification EP 3 265 493 B1, published January 10, 2024. Title: Method of Treating A Localized Fibrotic Disorder Using An IL-33 Antagonist. Applicant: 180 Therapeutics LP. The sequence listing filed with the application follows.

SEQUENCE LISTING (3 sequences)

SEQ ID NO: 1 - DNA, 21 bp, Homo sapiens
gccuugggucuacuaauaatt

SEQ ID NO: 2 - DNA, 21 bp, Homo sapiens
cggugacugucccaacuuutt

SEQ ID NO: 3 - DNA, 21 bp, Homo sapiens
guuacaccguggauugguatt